European Patent Application EP 4 371 564 A2, published May 22, 2024. Title: DESIGN OF BACTERIOPHAGE-BASED ARTIFICIAL VIRUSES FOR HUMAN GENOME REMODELING. Applicant: The Catholic University of America. Application WO PCT/IB2021/056248, filed July 21, 2021. The sequence listing filed with the application follows.

SEQUENCE LISTING (24 sequences)

SEQ ID NO: 1 - DNA, 120 bp, synthetic construct
  misc_feature 1..120: note = Synthetic: DNA template for AAVS1gRNA in vitro synthesis
  source 1..120: mol_type = other DNA
aagcaatacgactcactataggggccactagggacaggatgttttagagctagaaatagcaagttaaaataaggctagtccgttatcaacttgaaaaagtggcaccgagtcggtgctttt

SEQ ID NO: 2 - DNA, 20 bp, synthetic construct
  misc_feature 1..20: note = Synthetic: AAVS1-Cas9-gRNA1
  source 1..20: mol_type = other DNA
gtcccctccaccccacagtg

SEQ ID NO: 3 - DNA, 20 bp, synthetic construct
  misc_feature 1..20: note = Synthetic: AAVS1-Cas9-gRNA2
  source 1..20: mol_type = other DNA
ggggccactagggacaggat

SEQ ID NO: 4 - DNA, 20 bp, synthetic construct
  misc_feature 1..20: note = Synthetic: HBB-Cas9-gRNA
  source 1..20: mol_type = other DNA
agtctgccgttactgccctg

SEQ ID NO: 5 - DNA, 20 bp, synthetic construct
  misc_feature 1..20: note = Synthetic: ipIII-Cas9-gRNA
  source 1..20: mol_type = other DNA
ggcctttactacagaagctt

SEQ ID NO: 6 - DNA, 23 bp, synthetic construct
  misc_feature 1..23: note = Synthetic: ipI-Cpf1- gRNA1
  source 1..23: mol_type = other DNA
ttcagcaggagagataacgattg

SEQ ID NO: 7 - DNA, 23 bp, synthetic construct
  misc_feature 1..23: note = Synthetic: ipI-Cpf1-gRNA2
  source 1..23: mol_type = other DNA
taccattaccgaagctactctta

SEQ ID NO: 8 - DNA, 23 bp, synthetic construct
  misc_feature 1..23: note = Synthetic: ipII-Cpf1-gRNA1
  source 1..23: mol_type = other DNA
cttctaagttcggcatgtctatg

SEQ ID NO: 9 - DNA, 20 bp, synthetic construct
  misc_feature 1..20: note = Synthetic: ipII-Cpf1-gRNA2
  source 1..20: mol_type = other DNA
ttacggtctttatcgggcaa

SEQ ID NO: 10 - DNA, 23 bp, synthetic construct
  misc_feature 1..23: note = Synthetic: ipIII-Cpf1-gRNA1
  source 1..23: mol_type = other DNA
aagtcggaagcctttgtagctaa

SEQ ID NO: 11 - DNA, 23 bp, synthetic construct
  misc_feature 1..23: note = Synthetic: ipIII-Cpf1-gRNA2
  source 1..23: mol_type = other DNA
tgcttggcaaattcaagacctgc

SEQ ID NO: 12 - DNA, 20 bp, synthetic construct
  misc_feature 1..20: note = Synthetic: P1
  source 1..20: mol_type = other DNA
ctgccgtctctctcctgagt

SEQ ID NO: 13 - DNA, 20 bp, synthetic construct
  misc_feature 1..20: note = Synthetic: P2
  source 1..20: mol_type = other DNA
gtgggcttgtactcggtcat

SEQ ID NO: 14 - DNA, 20 bp, synthetic construct
  misc_feature 1..20: note = Synthetic: P3
  source 1..20: mol_type = other DNA
aaaactgacgcacggaggaa

SEQ ID NO: 15 - DNA, 20 bp, synthetic construct
  misc_feature 1..20: note = Synthetic: P4
  source 1..20: mol_type = other DNA
gtggattcgggtcacctctc

SEQ ID NO: 16 - protein, 1462 aa, synthetic construct
  REGION 1..1462: note = Synthetic: Cas9-Soc
PKKKRKVMDKKYSIGLDIGTNSVGWAVITDEYKVPSKKFKVLGNTDRHSIKKNLIGALLFDSGETAEATRLKRTARRRYTRRKNRICYLQEIFSNEMAKVDDSFFHRLEESFLVEEDKKHERHPIFGNIVDEVAYHEKYPTIHLRKKLVDSTDKADLRLIYLALAHMIKFRGHFLIEGDLNPDNSDVDKLFIQLVQTYNQLFEENPINASGVDAKAILSARLSKSRRLENLIAQLPGEKKNGLFGNLIALSLGLTPNFKSNFDLAEDAKLQLSKDTYDDDLDNLLAQIGDQYADLFLAAKNLSDAILLSDILRVNTEITKAPLSASMIKRYDEHHQDLTLLKALVRQQLPEKYKEIFFDQSKNGYAGYIDGGASQEEFYKFIKPILEKMDGTEELLVKLNREDLLRKQRTFDNGSIPHQIHLGELHAILRRQEDFYPFLKDNREKIEKILTFRIPYYVGPLARGNSRFAWMTRKSEETITPWNFEEVVDKGASAQSFIERMTNFDKNLPNEKVLPKHSLLYEYFTVYNELTKVKYVTEGMRKPAFLSGEQKKAIVDLLFKTNRKVTVKQLKEDYFKKIECFDSVEISGVEDRFNASLGTYHDLLKIIKDKDFLDNEENEDILEDIVLTLTLFEDREMIEERLKTYAHLFDDKVMKQLKRRRYTGWGRLSRKLINGIRDKQSGKTILDFLKSDGFANRNFMQLIHDDSLTFKEDIQKAQVSGQGDSLHEHIANLAGSPAIKKGILQTVKVVDELVKVMGRHKPENIVIEMARENQTTQKGQKNSRERMKRIEEGIKELGSQILKEHPVENTQLQNEKLYLYYLQNGRDMYVDQELDINRLSDYDVDHIVPQSFLKDDSIDNKVLTRSDKNRGKSDNVPSEEVVKKMKNYWRQLLNAKLITQRKFDNLTKAERGGLSELDKAGFIKRQLVETRQITKHVAQILDSRMNTKYDENDKLIREVKVITLKSKLVSDFRKDFQFYKVREINNYHHAHDAYLNAVVGTALIKKYPKLESEFVYGDYKVYDVRKMIAKSEQEIGKATAKYFFYSNIMNFFKTEITLANGEIRKRPLIETNGETGEIVWDKGRDFATVRKVLSMPQVNIVKKTEVQTGGFSKESILPKRNSDKLIARKKDWDPKKYGGFDSPTVAYSVLVVAKVEKGKSKKLKSVKELLGITIMERSSFEKNPIDFLEAKGYKEVKKDLIIKLPKYSLFELENGRKRMLASAGELQKGNELALPSKYVNFLYLASHYEKLKGSPEDNEQKQLFVEQHKHYLDEIIEQISEFSKRVILADANLDKVLSAYNKHRDKPIREQAENIIHLFTLTNLGAPAAFKYFDTTIDRKRYTSTKEVLDATLIHQSITGLYERIDLSQLGGDGGGGSRSGGYVNIKTFTHPAGEGKEVKGMEVSVPFEIYSNEHRIADAHYQTFPSEKAAYTVVTDAADWRTKNAAMFTPTPVSGHHHHHH

SEQ ID NO: 17 - protein, 1334 aa, synthetic construct
  REGION 1..1334: note = Synthetic: Cpf1-Soc
PKKKRKVMSKLEKFTNCYSLSKTLRFKAIPVGKTQENIDNKRLLVEDEKRAEDYKGVKKLLDRYYLSFINDVLHSIKLKNLNNYISLFRKKTRTEKENKELENLEINLRKEIAKAFKGNEGYKSLFKKDIIETILPEFLDDKDEIALVNSFNGFTTAFTGFFDNRENMFSEEAKSTSIAFRCINENLTRYISNMDIFEKVDAIFDKHEVQEIKEKILNSDYDVEDFFEGEFFNFVLTQEGIDVYNAIIGGFVTESGEKIKGLNEYINLYNQKTKQKLPKFKPLYKQVLSDRESLSFYGEGYTSDEEVEVFRNTLNKNSEIFSSIKKLEKLFKNFDEYSSAGIFVKNGPAISTISKDIFGEWNVIRDKWNAEYDDIHLKKKAVVTEKYEDDRRKSFKKIGSFSLEQLQEYADADLSVVEKLKEIIIQKVDEIYKVYGSSEKLFDADFVLEKSLKKNDAVVAIMKDLLDSVKSFENYIKAFFGEGKETNRDESFYGDFVLAYDILLKVDHIYDAIRNYVTQKPYSKDKFKLYFQNPQFMGGWDKDKETDYRATILRYGSKYYLAIMDKKYAKCLQKIDKDDVNGNYEKINYKLLPGPNKMLPKVFFSKKWMAYYNPSEDIQKIYKNGTFKKGDMFNLNDCHKLIDFFKDSISRYPKWSNAYDFNFSETEKYKDIAGFYREVEEQGYKVSFESASKKEVDKLVEEGKLYMFQIYNKDFSDKSHGTPNLHTMYFKLLFDENNHGQIRLSGGAELFMRRASLKKEELVVHPANSPIANKNPDNPKKTTTLSYDVYKDKRFSEDQYELHIPIAINKCPKNIFKINTEVRVLLKHDDNPYVIGIDRGERNLLYIVVVDGKGNIVEQYSLNEIINNFNGIRIKTDYHSLLDKKEKERFEARQNWTSIENIKELKAGYISQVVHKICELVEKYDAVIALEDLNSGFKNSRVKVEKQVYQKFEKMLIDKLNYMVDKKSNPCATGGALKGYQITNKFESFKSMSTQNGFIFYIPAWLTSKIDPSTGFVNLLKTKYTSIADSKKFISSFDRIMYVPEEDLFEFALDYKNFSRTDADYIKKWKLYSYGNRIRIFRNPKKNNVFDWEEVCLTSAYKELFNKYGINYQQGDIRALLCEQSDKAFYSSFMALMSLMLQMRNSITGRTDVDFLISPVKNSDGIFYDSRNYEAQENAILPKNADANGAYNIARKVLWAIGQFKKAEDEKLDKVKIAISNKEWLEYAQTSVKHAAAGGGGSGGGGSRSGGYVNIKTFTHPAGEGKEVKGMEVSVPFEIYSNEHRIADAHYQTFPSEKAAYTTVVTDAADWRTKNAAMFTPTPVSGLEHHHHHH

SEQ ID NO: 18 - protein, 742 aa, synthetic construct
  REGION 1..742: note = Synthetic: Cre-Hoc
MSNLLTVHQNLPALPVDATSDEVRKNLMDMFRDRQAFSEHTWKMLLSVCRSWAAWCKLNNRKWFPAEPEDVRDYLLYLQARGLAVKTIQQHLGQLNMLHRRSGLPRPSDSNAVSLVMRRIRKENVDAGERAKQALAFERTDFDQVRSLMENSDRCQDIRNLAFLGIAYNTLLRIAEIARIRVKDISRTDGGRMLIHIGRTKTLVSTAGVEKALSLGVTKLVERWISVSGVADDPNNYLFCRVRKNGVAAPSATSQLSTRALEGIFEATHRLIYGAKDDSGQRYLAWSGHSARVGAARDMARAGVSIPEIMQAGGWTNVNIVMNYIRNLDSETGAMVRLLEDGDGGSEFGGSGGSGGSGGSFTVDITPKTPTGVIDETKQFTATPSGQTGGGTITYAWSVDNVPQDGAEATFSYVLKGPAGQKTIKVVATNTLSEGGPETAEATTTITVKNKTQTTTLAVTPASPAAGVIGTPVQFTAALASQPDGASATYQWYVDDSQVGGETNSTFSYTPTTSGVKRIKCVAQVTATDYDALSVTSNEVSLTVNKKTMNPQVTLTPPSINVQQDASATFTANVTGAPEEAQITYSWKKDSSPVEGSTNVYTVDTSSVGSQTIEVTATVTAADYNPVTVTKTGNVTVTAKVAPEPEGELPYVHPLPHRSSAYIWCGWWVMDEIQKMTEEGKDWKTDDPDSKYYLHRYTLQKMMKDYPEVDVQESRNGYIIHKTALETGIIYTYPGSHHHHHH

SEQ ID NO: 19 - protein, 400 aa, synthetic construct
  REGION 1..400: note = Synthetic: RGD-Hoc
CDCRGDCFCSAMTFTVDITPKTPTGVIDETKQFTATPSGQTGGGTITYAWSVDNVPQDGAEATFSYVLKGPAGQKTIKVVATNTLSEGGPETAEATTTITVKNKTQTTTLAVTPASPAAGVIGTPVQFTAALASQPDGASATYQWYVDDSQVGGETNSTFSYTPTTSGVKRIKCVAQVTATDYDALSVTSNEVSLTVNKKTMNPQVTLTPPSINVQQDASATFTANVTGAPEEAQITYSWKKDSSPVEGSTNVYTVDTSSVGSQTIEVTATVTAADYNPVTVTKTGNVTVTAKVAPEPEGELPYVHPLPHRSSAYIWCGWWVMDEIQKMTEEGKDWKTDDPDSKYYLHRYTLQKMMKDYPEVDVQESRNGYIIHKTALETGIIYTYPKLAAALEHHHHHH

SEQ ID NO: 20 - protein, 90 aa, synthetic construct
  REGION 1..90: note = Synthetic: CTS-LacI-NLS
MKTYQEFIAEMKYVTLYDVAEYAGVSHQTVSRVVNQASHVSAKTREKVEAAMAELNYIPNRVAQQLAGKQSLLIKRPAATKKAGQAKKKK

SEQ ID NO: 21 - DNA, 6806 bp, synthetic construct
  misc_feature 1..6806: note = Synthetic: streptomycin-resistant plasmid DS-SPCas
  source 1..6806: mol_type = other DNA
accaggcacgcctaaccgtcagtgagattggatgagtgaacgatattgatcgagaagagccctgcgcagccgctgccgtgcctgcaggaagcaacggcccggagggtggcgggcaggacgcccgccataaactgccaggcatcaaattaagcagaaggccatcctgacggatggcctttttgcgtttctacaaactctgctagcttctagagcacagctaacaccacgtcgtccctatctgctgccctaggtctatgagtggttgctggataactttacgggcatgcataaggctcgtatgatatattcagggagaccacaacggtttccctctacaaataattttgtttaacttttactagaggaggaggcaaaaatggataagaaatactcaataggcttagatatcggcacaaatagcgtcggatgggcggtgatcactgatgaatataaggttccgtctaaaaagttcaaggttctgggaaatacagaccgccacagtatcaaaaaaaatcttataggggctcttttatttgacagtggagagacagcggaagcgactcgtctcaaacggacagctcgtagaaggtatacacgtcggaagaatcgtatttgttatctacaggagattttttcaaatgagatggcgaaagtagatgatagtttctttcatcgacttgaagagtcttttttggtggaagaagacaagaagcatgaacgtcatcctatttttggaaatatagtagatgaagttgcttatcatgagaaatatccaactatctatcatctgcgaaaaaaattggtagattctactgataaagcggatttgcgcttaatctatttggccttagcgcatatgattaagtttcgtggtcattttttgattgagggagatttaaatcctgataatagtgatgtggacaaactatttatccagttggtacaaacctacaatcaattatttgaagaaaaccctattaacgcaagtggagtagatgctaaagcgattctttctgcacgattgagtaaatcaagacgattagaaaatctcattgctcagctccccggtgagaagaaaaatggcttatttgggaatctcattgctttgtcattgggtttgacccctaattttaaatcaaattttgatttggcagaagatgctaaattacagctttcaaaagatacttacgatgatgatttagataatttattggcgcaaattggagatcaatatgctgatttgtttttggcagctaagaatttatcagatgctattttactttcagatatcctaagagtaaatactgaaataactaaggctcccctatcagcttcaatgattaaacgctacgatgaacatcatcaagacttgactcttttaaaagctttagttcgacaacaacttccagaaaagtataaagaaatcttttttgatcaatcaaaaaacggatatgcaggttatattgatgggggagctagccaagaagaattttataaatttatcaaaccaattttagaaaaaatggatggtactgaggaattattggtgaaactaaatcgtgaagatttgctgcgcaagcaacggacctttgacaacggctctattccccatcaaattcacttgggtgagctgcatgctattttgagaagacaagaagacttttatccatttttaaaagacaatcgtgagaagattgaaaaaatcttgacttttcgaattccttattatgttggtccattggcgcgtggcaatagtcgttttgcatggatgactcggaagtctgaagaaacaattaccccatggaattttgaagaagttgtcgataaaggtgcttcagctcaatcatttattgaacgcatgacaaactttgataaaaatcttccaaatgaaaaagtactaccaaaacatagtttgctttatgagtattttacggtttataacgaattgacaaaggtcaaatatgttactgaaggaatgcgaaaaccagcatttctttcaggtgaacagaagaaagccattgttgatttactcttcaaaacaaatcgaaaagtaaccgttaagcaattaaaagaagattatttcaaaaaaatagaatgttttgatagtgttgaaatttcaggagttgaagatagatttaatgcttcattaggtacctaccatgatttgctaaaaattattaaagataaagattttttggataatgaagaaaatgaagatatcttagaggatattgttttaacattgaccttatttgaagatagggagatgattgaggaaagacttaaaacatatgctcacctctttgatgataaggtgatgaaacagcttaaacgtcgccgttatactggttggggacgtttgtctcgaaaattgattaatggtattagggataagcaatctggcaaaacaatattagattttttgaaatcagatggttttgccaatcgcaattttatgcagctgatccatgatgatagtttgacatttaaagaagacattcaaaaagcacaagtgtctggacaaggcgatagtttacatgaacatattgcaaatttagctggtagccctgctattaaaaaaggtattttacagactgtaaaagttgttgatgaattggtcaaagtaatggggcggcataagccagaaaatatcgttattgaaatggcacgtgaaaatcagacaactcaaaagggccagaaaaattcgcgagagcgtatgaaacgaatcgaagaaggtatcaaagaattaggaagtcagattcttaaagagcatcctgttgaaaatactcaattgcaaaatgaaaagctctatctctattatctccaaaatggaagagacatgtatgtggaccaagaattagatattaatcgtttaagtgattatgatgtcgatcacattgttccacaaagtttccttaaagacgattcaatagacaataaggtcttaacgcgttctgataaaaatcgtggtaaatcggataacgttccaagtgaagaagtagtcaaaaagatgaaaaactattggagacaacttctaaacgccaagttaatcactcaacgtaagtttgataatttaacgaaagctgaacgtggaggtttgagtgaacttgataaagctggttttatcaaacgccaattggttgaaactcgccaaatcactaagcatgtggcacaaattttggatagtcgcatgaatactaaatacgatgaaaatgataaacttattcgagaggttaaagtgattaccttaaaatctaaattagtttctgacttccgaaaagatttccaattctataaagtacgtgagattaacaattaccatcatgcccatgatgcgtatctaaatgccgtcgttggaactgctttgattaagaaatatccaaaacttgaatcggagtttgtctatggtgattataaagtttatgatgttcgtaaaatgattgctaagtctgagcaagaaataggcaaagcaaccgcaaaatatttcttttactctaatatcatgaacttcttcaaaacagaaattacacttgcaaatggagagattcgcaaacgccctctaatcgaaactaatggggaaactggagaaattgtctgggataaagggcgagattttgccacagtgcgcaaagtattgtccatgccccaagtcaatattgtcaagaaaacagaagtacagacaggcggattctccaaggagtcaattttaccaaaaagaaattcggacaagcttattgctcgtaaaaaagactgggatccaaaaaaatatggtggttttgatagtccaacggtagcttattcagtcctagtggttgctaaggtggaaaaagggaaatcgaagaagttaaaatccgttaaagagttactagggatcacaattatggaaagaagttcctttgaaaaaaatccgattgactttttagaagctaaaggatataaggaagttaaaaaagacttaatcattaaactacctaaatatagtctttttgagttagaaaacggtcgtaaacggatgctggctagtgccggagaattacaaaaaggaaatgagctggctctgccaagcaaatatgtgaattttttatatttagctagtcattatgaaaagttgaagggtagtccagaagataacgaacaaaaacaattgtttgtggagcagcataagcattatttagatgagattattgagcaaatcagtgaattttctaagcgtgttattttagcagatgccaatttagataaagttcttagtgcatataacaaacatagagacaaaccaatacgtgaacaagcagaaaatattattcatttatttacgttgacgaatcttggagctcccgctgcttttaaatattttgatacaacaattgatcgtaaacgatatacgtctacaaaagaagttttagatgccactcttatccatcaatccatcactggtctttatgaaacacgcattgatttgagtcagctaggaggtgactgaccggctgataaatttctttgaatttctccttgattatttgttataaatgttataaaataatcttgttggaaccattcaaaacagcatagcaagttaaaataaggctagtccgttatcaacttgaaaaagtggcaccgagtcggtgctttttttgatacttctattctactctgactgcaaaccaaaaaaacaagcgctttcaaaacgcttgttttatcatttttagggaaattaatctcttaatccttttatcattctacatttaggcgctgccatcttgggacaatgaaaacgttagtcatggcgcgccttgacggctagctcagtcctaggtacagtgctagcttaattagtctacgaggttttagagctatgctgttttgaatggtcccaaaacctgcagacaagcccggccggcctaaggcgatgccccctcgacctcgatcagggaggcgttcaggacgactcacaaagaaagccgggcaatgcccggctttttccacgcctcctgggctgacttcaggtgctacatttgaagagataaattgcactgaaatctagagcggttcagtagaaaagatcaaaggatcttcttgagatcctttttttctgcgcgtaatcttttgccctgtaaacgaaaaaaccacctggggaggtggtttgatcgaaggttaagtcagttggggaactgcttaaccgtggtaactggctttcgcagagcacagcaaccaaatctgtccttccagtgtagccggactttggcgcacacttcaagagcaaccgcgtgtttagctaaacaaatcctctgcgaactcccagttaccaatggctgctgccagtggcgttttaccgtgcttttccgggttggactcaagtgaacagttaccggataaggcgcagcagtcgggctgaacggggagttcttgcttacagcccagcttggagcgaacgacctacaccgagccgagataccagtgtgtgagctatgagaaagcgccacacttcccgtaagggagaaaggcggaacaggtatccggtaaacggcagggtcggaacaggagagcgcaagagggagcgacccgccggaaacggtggggatctttaagtcctgtcgggtttcgcccgtactgtcagattcatggttgagcctcacggctcccacagatgcaccggaaaagcgtctgtttatgtgaactctggcaggagggcggagcctatggaaaaacgccaccggcgcggccctgctgttttgcctcacatgttagtcccctgcttatccacggaatctgtgggtaactttgtatgtgtccgcagcgcccgccgcagtctcacgcccggagcgtagcgaccgagtgagctagctatttgtttatttttctaaatacattcaaatatgtatccgctcatgagacaataaccctgataaatgcttcaataatattgaaaaaggaagagtatgagggaagcggtgatcgccgaagtatcgactcaactatcagaggtagttggcgtcatcgagcgccatctcgaaccgacgttgctggccgtacatttgtacggctccgcagtggatggcggcctgaagccacacagtgatattgatttgctggttacggtgaccgtaaggcttgatgaaacaacgcggcgagctttgatcaacgaccttttggaaacttcggcttcccctggagagagcgagattctccgcgctgtagaagtcaccattgttgtgcacgacgacatcattccgtggcgttatccagctaagcgcgaactgcaatttggagaatggcagcgcaatgacattcttgcaggtatcttcgagccagccacgatcgacattgatctggctatcttgctgacaaaagcaagagaacatagcgttgccttggtaggtccagcggcggaggaactctttgatccggttcctgaacaggatctatttgaggcgctaaatgaaaccttaacgctatggaactcgccgcccgactgggctggcgatgagcgaaatgtagtgcttacgttgtcccgcatttggtacagcgcagtaaccggcaaaatcgcgccgaaggatgtcgctgccgactgggcaatggagcgcctgccggcccagtatcagcccgtcatacttgaagctagacaggcttatcttggacaagaagaagatcgcttggcctcgcgcgcagatcagttggaagaatttgtccactacgtgaaaggcgagatcaccaaggtagtcggcaaataatgtctaacaattcgttcaagccgaggggccgcaagatccggccacgatgacccggtcgtcggttcagggcagggt

SEQ ID NO: 22 - protein, 445 aa, synthetic construct
  REGION 1..445: note = Synthetic: Cre-Soc
MSNLLTVHQNLPALPVDATSDEVRKNLMDMFRDRQAFSEHTWKMLLSVCRSWAAWCKLNNRKWFPAEPEDVRDYLLYLQARGLAVKTIQQHLGQLNMLHRRSGLPRPSDSNAVSLVMRRIRKENVDAGERAKQALAFERTDFDQVRSLMENSDRCQDIRNLAFLGIAYNTLLRIAEIARIRVKDISRTDGGRMLIHIGRTKTLVSTAGVEKALSLGVTKLVERWISVSGVADDPNNYLFCRVRKNGVAAPSATSQLSTRALEGIFEATHRLIYGAKDDSGQRYLAWSGHSARVGAARDMARAGVSIPEIMQAGGWTNVNIVMNYIRNLDSETGAMVRLLEDGDGGSEFGGSGGSGGSGGSGGYVNIKTFTHPAGEGKEVKGMEVSVPFEIYSNEHRIADAHYQTFPSEKAAYTTVVTDAADWRTKNAAMFTPTPVSGGSHHHHHH

SEQ ID NO: 23 - protein, 9 aa, unidentified
  REGION 1..9: note = synthetic construct
CDCRGDCFC

SEQ ID NO: 24 - protein, 7 aa, unidentified
  REGION 1..7: note = synthetic construct
PKKKRKV